European Patent Specification EP 3 752 644 B1, published July 16, 2025. Title: TUMOR MINIMAL RESIDUAL DISEASE STRATIFICATION. Applicant: VIB VZW KATHOLIEKE UNIVERSITEIT LEUVEN, K.U.LEUVEN R&D. The sequence listing filed with the application follows.

SEQUENCE LISTING (70 sequences)

SEQ ID NO: 1 - protein, 37 aa, Artificial Sequence
  37-residue amphipathic peptide
DWLKAFYDKVAEKLKEAFPDWAKAAYDKAAEKAKEAA

SEQ ID NO: 2 - DNA, 21 bp, Artificial Sequence
  siRNA
gaaccuauugauggauuaatt

SEQ ID NO: 3 - DNA, 21 bp, Artificial Sequence
  siRNA
ccuucacuaucaguuggaatt

SEQ ID NO: 4 - DNA, 21 bp, Artificial Sequence
  siRNA
gcaacauucaaguuaagcatt

SEQ ID NO: 5 - DNA, 58 bp, Artificial Sequence
  shRNA
ccgggaagttacatattaggccatactcgagtatggcctaatatgtaacttctttttg

SEQ ID NO: 6 - DNA, 58 bp, Artificial Sequence
  shRNA
ccggccgacgttaatctgaaaggaactcgagttcctttcagattaacgtcggtttttg

SEQ ID NO: 7 - DNA, 58 bp, Artificial Sequence
  shRNA
ccgggccataatcgacacatataaactcgagtttatatgtgtcgattatggctttttg

SEQ ID NO: 8 - DNA, 58 bp, Artificial Sequence
  shRNA
ccggcctgcttatccagaagacaatctcgagattgtcttctggataagcaggtttttg

SEQ ID NO: 9 - DNA, 58 bp, Artificial Sequence
  shRNA
ccggccattggtgatgagaaggcaactcgagttgccttctcatcaccaatggtttttg

SEQ ID NO: 10 - DNA, 57 bp, Artificial Sequence
  shRNA
ccgggcagatgaagatcatcgaaatctcgagatttcgatgatcttcatctgcttttt

SEQ ID NO: 11 - DNA, 57 bp, Artificial Sequence
  shRNA
ccggccgctgtcaaacatgtggttactcgagtaaccacatgtttgacagcggttttt

SEQ ID NO: 12 - DNA, 57 bp, Artificial Sequence
  shRNA
ccgggctggtttccaaacagaggatctcgagatcctctgtttggaaaccagcttttt

SEQ ID NO: 13 - DNA, 57 bp, Artificial Sequence
  shRNA
ccggcagcagttacaagccttcaaactcgagtttgaaggcttgtaactgctgttttt

SEQ ID NO: 14 - DNA, 57 bp, Artificial Sequence
  shRNA
ccggctatgaagaatacaccagcaactcgagttgctggtgtattcttcatagttttt

SEQ ID NO: 15 - DNA, 57 bp, Artificial Sequence
  shRNA
ccggcgggattggaaacatgaactactcgagtagttcatgtttccaatcccgttttt

SEQ ID NO: 16 - DNA, 57 bp, Artificial Sequence
  shRNA
ccgggagtcctaactgagctggtttctcgagaaaccagctcagttaggactcttttt

SEQ ID NO: 17 - DNA, 57 bp, Artificial Sequence
  shRNA
ccgggcctacaccaagcagaagtatctcgagatacttctgcttggtgtaggcttttt

SEQ ID NO: 18 - DNA, 57 bp, Artificial Sequence
  shRNA
ccggctatcagaagtgccttgtcatctcgagatgacaaggcacttctgatagttttt

SEQ ID NO: 19 - DNA, 57 bp, Artificial Sequence
  shRNA
ccgggcgagccattgtactctttaactcgagttaaagagtacaatggctcgcttttt

SEQ ID NO: 20 - DNA, 57 bp, Artificial Sequence
  shRNA
ccggctttaggttctttgctgcattctcgagaatgcagcaaagaacctaaagttttt

SEQ ID NO: 21 - DNA, 57 bp, Artificial Sequence
  shRNA
ccgggcggtctgcatgaaggaatttctcgagaaattccttcatgcagaccgcttttt

SEQ ID NO: 22 - DNA, 57 bp, Artificial Sequence
  shRNA
ccggcgaaagaaggagacccgttatctcgagataacgggtctccttctttcgttttt

SEQ ID NO: 23 - DNA, 57 bp, Artificial Sequence
  shRNA
ccggcgaaatcctctatgtcaacatctcgagatgttgacatagaggatttcgttttt

SEQ ID NO: 24 - DNA, 57 bp, Artificial Sequence
  shRNA
ccgggctgtgaagacgatgaagattctcgagaatcttcatcgtcttcacagcttttt

SEQ ID NO: 25 - DNA, 20 bp, artificial sequence
  Primer
catgtacatcatcgcccagt

SEQ ID NO: 26 - DNA, 19 bp, artificial sequence
  Primer
caccatcagccaggtcatt

SEQ ID NO: 27 - DNA, 21 bp, artificial sequence
  Primer
tcatccctgtctattgctcca

SEQ ID NO: 28 - DNA, 20 bp, artificial sequence
  Primer
tgttctgcttgcagctgttc

SEQ ID NO: 29 - DNA, 20 bp, artificial sequence
  Primer
gaccgggtgcccagcgagta

SEQ ID NO: 30 - DNA, 19 bp, artificial sequence
  Primer
cagccgggaccgacacagg

SEQ ID NO: 31 - DNA, 20 bp, artificial sequence
  Primer
atgctggaagggttcttctc

SEQ ID NO: 32 - DNA, 20 bp, artificial sequence
  Primer
tttcattctggtgtgccatc

SEQ ID NO: 33 - DNA, 20 bp, artificial sequence
  Primer
ctgcctgcttatccagatcc

SEQ ID NO: 34 - DNA, 20 bp, artificial sequence
  Primer
cctcacacttgaggctgatg

SEQ ID NO: 35 - DNA, 20 bp, artificial sequence
  Primer
accttggaaagtgccttgac

SEQ ID NO: 36 - DNA, 21 bp, artificial sequence
  Primer
ctcacagtgcacaatactgac

SEQ ID NO: 37 - DNA, 23 bp, artificial sequence
  Primer
ccctaccactgggtacagatgga

SEQ ID NO: 38 - DNA, 23 bp, artificial sequence
  Primer
cttcaagacacagacagccagga

SEQ ID NO: 39 - DNA, 20 bp, artificial sequence
  Primer
cctcttcatcttgggctttg

SEQ ID NO: 40 - DNA, 19 bp, artificial sequence
  Primer
agcccctcctactccacag

SEQ ID NO: 41 - DNA, 20 bp, artificial sequence
  Primer
tggggcacctggagttaatg

SEQ ID NO: 42 - DNA, 20 bp, artificial sequence
  Primer
atcttaaagtcccgtccggc

SEQ ID NO: 43 - DNA, 19 bp, artificial sequence
  Primer
cgaatgcctcaatgcgtct

SEQ ID NO: 44 - DNA, 20 bp, artificial sequence
  Primer
cccatttttcgatttggctc

SEQ ID NO: 45 - DNA, 21 bp, artificial sequence
  Primer
cccttgaggcctacaccaagc

SEQ ID NO: 46 - DNA, 21 bp, artificial sequence
  Primer
cacacctgcccaggggtcatc

SEQ ID NO: 47 - DNA, 22 bp, artificial sequence
  Primer
tccaccaggcagcaagaatacg

SEQ ID NO: 48 - DNA, 22 bp, artificial sequence
  Primer
ggagttgctacggaaaccactg

SEQ ID NO: 49 - DNA, 26 bp, artificial sequence
  Primer
gggaaatgggaggggtgcaaaagagg

SEQ ID NO: 50 - DNA, 26 bp, artificial sequence
  Primer
ttgcgtgagtgtggatgggattggtg

SEQ ID NO: 51 - DNA, 19 bp, artificial sequence
  Primer
ccagtacccgcacctgcac

SEQ ID NO: 52 - DNA, 21 bp, artificial sequence
  Primer
ctttcgttcagcagcctccag

SEQ ID NO: 53 - DNA, 25 bp, artificial sequence
  Primer
cattgttatgctggaaatgctagaa

SEQ ID NO: 54 - DNA, 23 bp, artificial sequence
  Primer
ggcttgctgtatgtggtacttgg

SEQ ID NO: 55 - DNA, 20 bp, artificial sequence
  Primer
ggctggaccgagagagtttc

SEQ ID NO: 56 - DNA, 20 bp, artificial sequence
  Primer
tgctgttgtgcttaacccct

SEQ ID NO: 57 - DNA, 24 bp, artificial sequence
  Primer
ggtggtcgctaggtatgaataacc

SEQ ID NO: 58 - DNA, 19 bp, artificial sequence
  Primer
tccaccttcgatgtcggaa

SEQ ID NO: 59 - DNA, 19 bp, artificial sequence
  Primer
tgcacctacggatgcactg

SEQ ID NO: 60 - DNA, 20 bp, artificial sequence
  Primer
cgatggacgggatcttaggc

SEQ ID NO: 61 - DNA, 24 bp, artificial sequence
  Primer
gtggtagcaccttcaaagaaatcc

SEQ ID NO: 62 - DNA, 22 bp, artificial sequence
  Primer
gcaacttcctcacgggtgtgtc

SEQ ID NO: 63 - DNA, 20 bp, artificial sequence
  Primer
atggcaaatagaggaagcgg

SEQ ID NO: 64 - DNA, 21 bp, artificial sequence
  Primer
tggagaatagatcgaagcaag

SEQ ID NO: 65 - DNA, 21 bp, artificial sequence
  Primer
aatctgtcatgctggtctgcc

SEQ ID NO: 66 - DNA, 20 bp, artificial sequence
  Primer
aggagatttgtttggcgtgc

SEQ ID NO: 67 - DNA, 19 bp, artificial sequence
  Primer
atttgggtcgcggttcttg

SEQ ID NO: 68 - DNA, 21 bp, artificial sequence
  Primer
tgccttgacattctcgatggt

SEQ ID NO: 69 - DNA, 24 bp, artificial sequence
  Primer
acttttggtacattgtggcttcaa

SEQ ID NO: 70 - DNA, 20 bp, artificial sequence
  Primer
ccgccaggacaaaccagtat